European Patent Specification EP 4 416 291 B1, published January 21, 2026. Title: PROCEDE DE PURIFICATION D'UNE PROTEINE D'INTERET ET MOYENS POUR SA MISE EN OEUVRE. Applicant: UNIVERSITE GRENOBLE ALPES. Application EP. The sequence listing filed with the application follows.

SEQUENCE LISTING (46 sequences)

SEQ ID NO: 1 - protein, 488 aa, Schizosaccharomyces pombe
MSNTNFSTSRSSKSIPELPNLEALRSLWPPPSLNESGDTRSVWTTHTGEPVASSVLSTSGSNNFSSPLKRPAPESHDAPIGRRLMVDDPRLIKHGKYDFSRHCTDYGHSYEWPYFRSLRRESMLYHTSGSYPESQPPYSSYSTDAPHYYHAGSESSAYYDSRSRLHGIQPPPKRRTLSPPPRRLADPVVVGSSRYVEEEVYRRPPYTLASEVPSSASAYQAGYSSYPVRSSPQLSHEDTRHGIASSGSTRYPFVPANTRASHSPSLLEPYAHSLPSSVAPVGAYPEKSSYLLSNSSNDSASRKEKPKARASTPPPLNFSRASEHRNEKGERISMINPRVVLDENGISHRSRYFIMLCDNETAIAHAKKTSIWAVKKDSSKRISDAYKKASVYFIFVAQQTYNALGYAQVVSDLNSTELPFWSDSSHAGGVRIKWIKTCNLFSAEISEIVSHMDHGSEARDGMEMMYDEGSRLCTLINYAIMKRIGRDR

SEQ ID NO: 2 - DNA, 1467 bp, Schizosaccharomyces pombe
  source 1..1467: mol_type = genomic DNA
atgtcaaacacaaacttctctacttctaggtcatcaaagtccattccggaacttccaaatttggaagctctgcgaagcctgtggcctccaccgtcattgaacgaatcgggcgatactagaagcgtatggactactcataccggagagcctgttgcgtcaagtgttctatctacttcaggttcaaacaacttttcttcacctctgaaaagacctgcaccagagtcacatgacgctcctatcggtagaagattgatggtagatgatccccgcttaattaaacatggtaaatatgattttagcaggcattgcactgactatggtcactcctacgaatggccttattttcgatcccttcgtcgtgagtctatgctttatcacacttcgggatcttatccagaaagtcagcctccttactcttcttattcaactgatgctccacattattatcatgcaggttcggaatcctctgcttactatgatagccgttctcgtttgcatggcatacaacctcctcccaagcgacgcacacttagtcctccccctagacggcttgcggacccagtggttgttggaagttctcgttatgttgaagaagaagtatacagaaggcctccttacactttagcttctgaagttccttcatccgcttcagcataccaagctggttactcttcctatcctgttcgatcttccccccaactttctcatgaagacactcgtcatggtattgcaagcagtggttcaacaaggtatccttttgtacctgctaatactcgtgcatctcactcccctagtttgcttgaaccttatgctcactcccttccctcttcggtcgcgccagttggagcttatcctgagaaatcttcttacctgctttctaattccagcaatgatagtgcctcaagaaaagaaaaacccaaagctcgtgcatctacgcctcctccattaaatttttccagagcaagcgaacatagaaatgagaagggggaacgcatttcgatgattaatccccgagttgttcttgacgaaaatggaatttcacaccgctcccgttattttattatgctatgtgacaacgagactgccattgctcatgctaaaaaaacttctatttgggcagtcaagaaagattcttccaaaagaatttctgatgcatataagaaagccagtgtttattttatttttgtggctcagcaaacgtacaatgctttaggatatgctcaggtagtcagcgacctaaatagcaccgaactgcccttttggtcagatagctcgcatgctggaggtgttcgcatcaagtggattaaaacttgcaatctgttttctgctgaaatttctgaaattgttagccacatggatcatgggtctgaagctagagatggcatggaaatgatgtatgatgaaggcagcagactttgtacgttgattaactatgctataatgaagcgaattggaagagaccgttga

SEQ ID NO: 3 - protein, 479 aa, Schizosaccharomyces japonicus
MSNSNASLQAAAIPSMEALRTLWRNIAPSTSGDSQEARSVWAKHPNDPTVPAAAPAAAGLFSSPLKRGAPDSKEYMDRHVLSEPVSVSSATVYDFYRHCTDYGHSYDWPYFRSLRRELAYRNSVDAAPYPPYRPEPSPRYAVPPYGQRSPTNYPMRYEESLQSAGQPPLKRRTLLSPHLSGMNSRLMMPSRYEDEYYTRPYNYGKAPAQASSFQSTMHSNGYTPARPESVPESAGIHGYHPMRQDAGDSPLFSEPTAHTEGYRDFDPLHGKFAPPSSHSYGIEPYDHKAEPRREKPKTRAPTPPPLDFEHAHEYRNEKGERVSMINPRVILDENGISHRSRYFIMLVDNETAISHAKRSSVWSLKQNYANAISEAYKQEANVYFIFINAKSYNALGYAQLTSDVGTVAKPFWADTTYTNGVNVKWIKTCNLYSNEISEIVSRMDHGARARDGQEMMYDEGSRLCTLINSAIMKRIGRDR

SEQ ID NO: 4 - DNA, 1440 bp, Schizosaccharomyces japonicus
  source 1..1440: mol_type = genomic DNA
atgtcgaattccaatgcttcactgcaagcggctgccataccgagtatggaggcgttaagaacgctatggcgtaacatagctccttccacttccggcgattcacaagaggcccggagtgtttgggctaagcatccaaatgatcctacggttcctgctgctgctccagctgccgcaggtcttttttcctctccattgaaacgcggtgctcctgattcaaaagagtatatggatcgtcatgtgctttcagagcctgtttctgtgagcagtgctactgtgtatgacttctaccgtcactgcactgattacggccattcttatgattggccctacttccgttcattgcgtcgcgagttggcataccgcaattctgtcgacgctgctccttatcctccgtatcgcccagaacccagtccccgctacgcagtacctccgtatggtcaacgttctccgacaaattatcccatgcgttatgaagagtctttgcagtctgcaggacagcccccgctaaaacgtcgtactttattaagtccacatttaagtggcatgaactctcggttaatgatgccttcacggtatgaagatgagtattacacgagaccttataattatggtaaggctcctgcccaagcgtcctcttttcaaagtaccatgcattccaatggctacactcctgcacgaccagaaagtgtcccggaatcagctggaatacatggataccaccctatgcggcaggatgctggcgattcaccattgttttcggaaccaactgctcatactgaagggtatcgcgatttcgatcctttacacggaaagtttgctcccccgtcctctcattcgtatggcatcgagccttatgaccataaagccgaacctcgtcgtgaaaaacccaaaacacgagcacctacaccccctccgttggattttgagcatgctcacgaatatcgcaatgaaaagggtgaacgtgtctccatgatcaatccacgtgttatccttgatgaaaatggaatctcacataggtcgcggtacttcatcatgctggtggataatgaaacagcaattagtcatgccaaacgaagttctgtttggagtcttaaacaaaattatgcgaacgctatcagcgaagcttacaagcaagaagcaaatgtctattttattttcatcaatgccaagtcctataatgcactggggtatgctcagcttacttctgatgtcgggactgttgcgaaaccgttttgggcagataccacatacactaatggtgtaaatgtcaagtggattaaaacgtgtaacttgtattcaaacgaaatttcagaaattgtgagccgcatggatcacggtgctcgggctagagatggtcaagaaatgatgtacgacgaaggaagtcgtctctgtaccttgatcaattcggcgattatgaaacgtattggtagagatcgttga

SEQ ID NO: 5 - protein, 480 aa, Schizosaccharomyces octosporus
MSNTNFNPQSSKQLPELPNLEVLRSLWPSQPSNEPNDSRSVWSNRPAEPVHVLSNPAANSFTSPLKRPAPDSREAPMGRRIMVDDPRLAKAVKYDFTRHCTDYGHSYEWPYFRSVRRESLMYGPPPAAVPPESPVFPPYSAEPASLQPKYYPPESDIPATFYDRARFGLQPPSKRRTLSPPPRRVVDPYGPHFVEEDPYSKSSYALAGDRPPLSAPMYPVGYPPYSAKAPSQIAADDFRGTASRYPLTASDVRASHSPGLIDPYTHRPVADVAYADRSHYAMNAEPYSAPPPRKEKPKPRAPTPPPLNFARASEYRNDKGERISMINPRVILDENGISSRSRYFIMLCDNETAISHAKKTSIWAVKHDAASRVSDAYKNASIYFIFIAKPTNNALGYAQVVSDLNSAELPFWADNATYAGGVRVKWIKTCNLFSAEISDIVGRMNHGATARDGMEMMYDEGCRLCILVNSAIMKRIGRDR

SEQ ID NO: 6 - DNA, 1443 bp, Schizosaccharomyces octosporus
  source 1..1443: mol_type = genomic DNA
atgtcaaacacaaactttaatcctcagtcttctaaacaattacctgaactcccaaacttggaggtattacgaagcttgtggccttctcaaccatcaaacgaacctaatgactccaggagtgtctggtctaacagaccggcggagcctgtgcatgtgctatcaaatcctgctgcgaatagttttacttctcctttaaaacgtccagctcctgattctcgtgaagctcctatgggaagaagaattatggttgatgatccacgcttagcgaaagctgtgaagtacgattttacccggcactgtacggattatggtcattcttatgaatggccttattttcgttctgttcgtcgtgaatcgttgatgtatggtccaccacctgctgctgttcctcctgaatctcctgtttttccaccctattctgctgaaccagctagcctacaacccaaatactatccacccgagtctgatattcccgccacattttatgatcgtgctcgttttggactgcagcccccttcaaaacgtagaacattgagtcctcctccaagaagagttgttgatccatatggccctcactttgttgaggaggatccatactcaaaatcctcttacgcattggctggggatcgtcctcctttatcagcccccatgtatcctgttggctatcctccgtatagtgcgaaagctccttcccaaatagctgctgatgattttcgtgggactgctagtagatatcctttgacggctagtgacgttcgggcttctcattctcctggactcattgatccatatactcatcgtcctgttgcagacgttgcttatgcggatcgttctcattatgctatgaatgcagagccttattcggctcctcctcctagaaaggaaaaaccaaagccacgtgctcctacacctcctccattaaattttgctagagccagtgagtacagaaatgacaaaggtgaacggatatctatgatcaatcctcgtgtaattcttgatgaaaatggaatatctagccgctctcgttattttataatgctttgtgataacgagacggctatttctcatgcaaagaaaacgtccatttgggctgtaaagcacgatgcagcatcccgtgtatcagatgcttacaagaatgctagtatttatttcatttttattgctaagccaacaaacaacgctcttggctatgctcaagttgttagtgatttgaatagcgcggagcttccgttttgggcagataatgctacctatgctggaggcgttcgcgtgaagtggattaaaacttgcaatcttttctctgccgagatatctgatatcgttggacgaatgaaccatggagcaaccgctagagatggaatggaaatgatgtacgatgaaggttgccgtctttgcatattggttaactcggccatcatgaagcgaatcggtcgtgatcggtaa

SEQ ID NO: 7 - protein, 479 aa, Schizosaccharomyces cryophilus
MSNTNFNSQSSKQLPELPNLEVLRSLWPSQPSNESNDSRSVWSSRPAEPVHVLSNPTANSFTSPLKRPAPDSREAPIGRRIMIDDPRLAKPVKYDFTRHCTDYGHSYEWPYFRSVRRESLMYGPPSAVPPESPVFPPYPPESATLQSKYYPAQSDAPAAYYDRARFELQPPSKRRTLSPPPRRIVDPYGPRFTEDDPYSKSPYAMAGDRPPLSAPMYPVGYPPYGAKASSQLGADDLRGTTSRYPLMASDVRASHSPSLIDPYAHRSVADVPYADHPHYSVNAEPYSAPPPRKEKPKPRAPTPPPLNFARASEYRNDKGERISMINPRVILDESGISHRSRYFIMLCDNETAIAHAKKTSIWAVKHEAASRVSDAYKKASIYFIFIAKPTNNALGYAQVVSDLNSAELPFWADNATYAGGVRVKWIKTCNLFSAEISDIVGRMNHGMTAKDGMEMMYDEGCRLCILVNSAIMKRIGRDR

SEQ ID NO: 8 - DNA, 1440 bp, Schizosaccharomyces cryophilus
  source 1..1440: mol_type = genomic DNA
atgtcaaacacaaactttaattctcagtcttctaaacaattacctgaactcccaaacttggaggttttgcgaagcttatggccttctcaaccgtcaaacgaatctaatgactctagaagtgtctggtcaagcagaccagcggaacccgtccatgtactttcaaatcctactgcgaatagttttacttctcctttaaaaagaccggctcccgattctcgtgaggcccccattggaagaagaattatgattgatgatccacgcttagcgaagccagtgaaatatgattttactcgccattgtactgattatggccattcttatgagtggccttactttcgctctgttcgtcgtgaatcgttaatgtatggaccgccttctgctgttcctcctgagtctcctgttttcccaccatatcctcccgagtcagctacgctgcaatccaaatactatccagcccaatctgatgcacctgccgcgtattatgatcgcgctcgttttgaattgcaacctccttcaaagcgaagaacattgagtcctccaccaaggagaatcgttgacccatatggtcctcgttttactgaggatgatccctactcaaaatcaccatatgcaatggctggcgatcgtcctccattatcagctcccatgtatcctgttggctatcctccgtatggtgcgaaagcttcctctcagcttggtgctgatgatttgcgtggtaccactagtagatatcccttgatggctagtgatgttcgtgcttctcattctcctagccttattgacccttatgcccatcgttctgttgcagatgttccttatgcggatcaccctcattactcagtgaacgctgagccttattcagcacctcctcccagaaaggaaaaacctaagccgcgtgctcccactccccctccgctaaattttgcgagagcaagtgaatatagaaatgacaaaggcgaacggatatctatgattaaccctcgtgtgattcttgacgaaagtggaatttcacatcgctctcgttattttattatgctttgtgacaacgaaacagcgattgcccatgcaaagaaaacctctatttgggctgtaaagcacgaagcagcttctcgtgtatctgatgcatataagaaggctagtatctattttatttttattgcaaagccgacaaataatgctcttggttatgctcaagtcgtgagtgatttgaacagtgcagaactccctttttgggcagataatgctacatacgccggaggcgttcgtgtgaaatggattaaaacttgcaatcttttctctgctgaaatctctgatatcgttggacgaatgaatcacggaatgactgctaaagatggaatggaaatgatgtacgacgagggatgccgcctttgtattttggttaactcggccatcatgaagcgaattggacgtgatcggtaa

SEQ ID NO: 9 - protein, 173 aa, Schizosaccharomyces pombe
LNFSRASEHRNEKGERISMINPRVVLDENGISHRSRYFIMLCDNETAIAHAKKTSIWAVKKDSSKRISDAYKKASVYFIFVAQQTYNALGYAQVVSDLNSTELPFWSDSSHAGGVRIKWIKTCNLFSAEISEIVSHMDHGSEARDGMEMMYDEGSRLCTLINYAIMKRIGRDR

SEQ ID NO: 10 - protein, 174 aa, Schizosaccharomyces japonicus
LDFEHAHEYRNEKGERVSMINPRVILDENGISHRSRYFIMLVDNETAISHAKRSSVWSLKQNYANAISEAYKQEANVYFIFINAKSYNALGYAQLTSDVGTVAKPFWADTTYTNGVNVKWIKTCNLYSNEISEIVSRMDHGARARDGQEMMYDEGSRLCTLINSAIMKRIGRDR

SEQ ID NO: 11 - protein, 174 aa, Schizosaccharomyces octosporus
LNFARASEYRNDKGERISMINPRVILDENGISSRSRYFIMLCDNETAISHAKKTSIWAVKHDAASRVSDAYKNASIYFIFIAKPTNNALGYAQVVSDLNSAELPFWADNATYAGGVRVKWIKTCNLFSAEISDIVGRMNHGATARDGMEMMYDEGCRLCILVNSAIMKRIGRDR

SEQ ID NO: 12 - protein, 174 aa, Schizosaccharomyces cryophilus
LNFARASEYRNDKGERISMINPRVILDESGISHRSRYFIMLCDNETAIAHAKKTSIWAVKHEAASRVSDAYKKASIYFIFIAKPTNNALGYAQVVSDLNSAELPFWADNATYAGGVRVKWIKTCNLFSAEISDIVGRMNHGMTAKDGMEMMYDEGCRLCILVNSAIMKRIGRDR

SEQ ID NO: 13 - protein, 11 aa, synthetic construct
  REGION 1..11: note = Domain 2 of Mmi1 of Schizosaccharomyces
  SITE 5: note = MISC_FEATURE - Xaa represents threonine, serine or alanine
  SITE 6: note = MISC_FEATURE - Xaa represents threonine, arginine, lysine or serine
  SITE 7: note = MISC_FEATURE - Xaa represents histidine or arginine
  SITE 8: note = MISC_FEATURE - Xaa represents threonine or proline
  SITE 9: note = MISC_FEATURE - Xaa represents glycine, alanine or arginine
  SITE 10: note = MISC_FEATURE - Xaa represents glutamic acid or aspartic acid
RSVWXXXXXXP

SEQ ID NO: 14 - protein, 19 aa, synthetic construct
  REGION 1..19: note = Domain 3 of Mmi1 of Schizosaccharomyces
  SITE 2: note = MISC_FEATURE - Xaa represents serine or threonine
  SITE 8: note = MISC_FEATURE - Xaa represents proline or glycine
  SITE 11: note = MISC_FEATURE - Xaa represents glutamic acid or aspartic acid
  SITE 13: note = MISC_FEATURE - Xaa represents histidine, arginine or lysine
  SITE 14: note = MISC_FEATURE - Xaa represents aspartic acid or glutamic acid
  SITE 15: note = MISC_FEATURE - Xaa represents alanine or tyrosine
  SITE 16: note = MISC_FEATURE - Xaa is null or represents proline
  SITE 17: note = MISC_FEATURE - Xaa represents isoleucine or methionine
  SITE 18: note = MISC_FEATURE - Xaa represents glycine or aspartic acid
FXSPLKRXAPXSXXXXXXR

SEQ ID NO: 15 - protein, 29 aa, synthetic construct
  REGION 1..29: note = Domain 4 of Mmi1 of Schizosaccharomyces
  SITE 4: note = MISC_FEATURE - Xaa represents serine, threonine or tyrosine
  SITE 15: note = MISC_FEATURE - Xaa represents glutamic acid or aspartic acid
  SITE 22: note = MISC_FEATURE - Xaa represents leucine or valine
  SITE 26: note = MISC_FEATURE - Xaa is null or represents serine
  SITE 27: note = MISC_FEATURE - Xaa represents leucine or methionine
  SITE 28: note = MISC_FEATURE - Xaa represents arginine, leucine or methionine
YDFXRHCTDYGHSYXWPYFRSXRREXXXY

SEQ ID NO: 16 - protein, 12 aa, synthetic construct
  REGION 1..12: note = Domain 5 of Mmi1 of Schizosaccharomyces
  SITE 4: note = MISC_FEATURE - Xaa represents proline, serine or leucine
  SITE 10: note = MISC_FEATURE - Xaa represents serine or leucine
  SITE 11: note = MISC_FEATURE - Xaa represents proline or serine
QPPXKRRTLXXP

SEQ ID NO: 17 - protein, 14 aa, synthetic construct
  REGION 1..14: note = Domain 6 of Mmi1 of Schizosaccharomyces
  SITE 1: note = MISC_FEATURE - Xaa represents arginine or aspartic acid
  SITE 3: note = MISC_FEATURE - Xaa represents serine or glycine
  SITE 4: note = MISC_FEATURE - Xaa represents histidine or aspartic acid
  SITE 7: note = MISC_FEATURE - Xaa represents serine, glycine or leucine
  SITE 8: note = MISC_FEATURE - Xaa represents leucine or phenylalanine
  SITE 9: note = MISC_FEATURE - Xaa represents leucine, isoleucine or serine
  SITE 10: note = MISC_FEATURE - Xaa represents glutamic acid or aspartic acid
  SITE 12: note = MISC_FEATURE - Xaa represents tyrosine or threonine
  SITE 13: note = MISC_FEATURE - Xaa represents alanine or threonine
XAXXSPXXXXPXXH

SEQ ID NO: 18 - protein, 14 aa, synthetic construct
  REGION 1..14: note = Domain 7 of Mmi1 of Schizosaccharomyces
  SITE 2: note = MISC_FEATURE - Xaa represents lysine or arginine
  SITE 7: note = MISC_FEATURE - Xaa represents alanine, proline or threonine
  SITE 10: note = MISC_FEATURE - Xaa represents serine or proline
RXEKPKXRAXTPPP

SEQ ID NO: 19 - protein, 11 aa, Schizosaccharomyces pombe
RSVWTTHTGEP

SEQ ID NO: 20 - protein, 19 aa, Schizosaccharomyces pombe
FSSPLKRPAPESHDAPIGR

SEQ ID NO: 21 - protein, 29 aa, Schizosaccharomyces pombe
YDFSRHCTDYGHSYEWPYFRSLRRESMLY

SEQ ID NO: 22 - protein, 12 aa, Schizosaccharomyces pombe
QPPPKRRTLSPP

SEQ ID NO: 23 - protein, 14 aa, Schizosaccharomyces pombe
RASHSPSLLEPYAH

SEQ ID NO: 24 - protein, 14 aa, Schizosaccharomyces pombe
RKEKPKARASTPPP

SEQ ID NO: 25 - protein, 458 aa, Schizosaccharomyces pombe
PSLNESGDTRSVWTTHTGEPVASSVLSTSGSNNFSSPLKRPAPESHDAPIGRRLMVDDPRLIKHGKYDFSRHCTDYGHSYEWPYFRSLRRESMLYHTSGSYPESQPPYSSYSTDAPHYYHAGSESSAYYDSRSRLHGIQPPPKRRTLSPPPRRLADPVVVGSSRYVEEEVYRRPPYTLASEVPSSASAYQAGYSSYPVRSSPQLSHEDTRHGIASSGSTRYPFVPANTRASHSPSLLEPYAHSLPSSVAPVGAYPEKSSYLLSNSSNDSASRKEKPKARASTPPPLNFSRASEHRNEKGERISMINPRVVLDENGISHRSRYFIMLCDNETAIAHAKKTSIWAVKKDSSKRISDAYKKASVYFIFVAQQTYNALGYAQVVSDLNSTELPFWSDSSHAGGVRIKWIKTCNLFSAEISEIVSHMDHGSEARDGMEMMYDEGSRLCTLINYAIMKRIGRDR

SEQ ID NO: 26 - protein, 11 aa, Schizosaccharomyces japonicus
RSVWAKHPNDP

SEQ ID NO: 27 - protein, 18 aa, Schizosaccharomyces japonicus
FSSPLKRGAPDSKEYMDR

SEQ ID NO: 28 - protein, 28 aa, Schizosaccharomyces japonicus
YDFYRHCTDYGHSYDWPYFRSLRRELAY

SEQ ID NO: 29 - protein, 12 aa, Schizosaccharomyces japonicus
QPPLKRRTLLSP

SEQ ID NO: 30 - protein, 14 aa, Schizosaccharomyces japonicus
DAGDSPLFSEPTAH

SEQ ID NO: 31 - protein, 14 aa, Schizosaccharomyces japonicus
RREKPKTRAPTPPP

SEQ ID NO: 32 - protein, 11 aa, Schizosaccharomyces octosporus
RSVWSNRPAEP

SEQ ID NO: 33 - protein, 19 aa, Schizosaccharomyces octosporus
FTSPLKRPAPDSREAPMGR

SEQ ID NO: 34 - protein, 29 aa, Schizosaccharomyces octosporus
YDFTRHCTDYGHSYEWPYFRSVRRESLMY

SEQ ID NO: 35 - protein, 12 aa, Schizosaccharomyces octosporus
QPPSKRRTLSPP

SEQ ID NO: 36 - protein, 14 aa, Schizosaccharomyces octosporus
RASHSPGLIDPYTH

SEQ ID NO: 37 - protein, 14 aa, Schizosaccharomyces octosporus
RKEKPKPRAPTPPP

SEQ ID NO: 38 - protein, 11 aa, Schizosaccharomyces cryophilus
RSVWSSRPAEP

SEQ ID NO: 39 - protein, 19 aa, Schizosaccharomyces cryophilus
FTSPLKRPAPDSREAPIGR

SEQ ID NO: 40 - protein, 29 aa, Schizosaccharomyces cryophilus
YDFTRHCTDYGHSYEWPYFRSVRRESLMY

SEQ ID NO: 41 - protein, 12 aa, Schizosaccharomyces cryophilus
QPPSKRRTLSPP

SEQ ID NO: 42 - protein, 14 aa, Schizosaccharomyces cryophilus
RASHSPSLIDPYAH

SEQ ID NO: 43 - protein, 14 aa, Schizosaccharomyces cryophilus
RKEKPKPRAPTPPP

SEQ ID NO: 44 - DNA, 519 bp, Schizosaccharomyces pombe
  source 1..519: mol_type = genomic DNA
aatttttccagagcaagcgaacatagaaatgagaagggggaacgcatttcgatgattaatccccgagttgttcttgacgaaaatggaatttcacaccgctcccgttattttattatgctatgtgacaacgagactgccattgctcatgctaaaaaaacttctatttgggcagtcaagaaagattcttccaaaagaatttctgatgcatataagaaagccagtgtttattttatttttgtggctcagcaaacgtacaatgctttaggatatgctcaggtagtcagcgacctaaatagcaccgaactgcccttttggtcagatagctcgcatgctggaggtgttcgcatcaagtggattaaaacttgcaatctgttttctgctgaaatttctgaaattgttagccacatggatcatgggtctgaagctagagatggcatggaaatgatgtatgatgaaggcagcagactttgtacgttgattaactatgctataatgaagcgaattggaagagaccgttga

SEQ ID NO: 45 - RNA, 18 nt, synthetic construct
  misc_feature 1..18: note = Substrate for Mmi1 binding
  misc_feature 1: note = Biotinylation
  source 1..18: mol_type = other RNA
ggatccttaaacagatct

SEQ ID NO: 46 - RNA, 18 nt, synthetic construct
  misc_feature 1..18: note = Negative control for Mmi1 binding
  misc_feature 1: note = Biotinylation
  source 1..18: mol_type = other RNA
ggatccctaaacagatct